European Patent Application EP 4 410 311 A1, published August 7, 2024. Title: Coiled-Coil Fusion Protein. Applicant: NBIOS Inc. The sequence listing filed with the application follows.

SEQUENCE LISTING (10 sequences)

SEQ ID NO: 1 - protein, 34 aa, synthetic construct
  REGION 1..34: note = MBD2_wild type
KAFIVTDEDIRKQEERVQQVRKKLEEALMADILS

SEQ ID NO: 2 - protein, 34 aa, synthetic construct
  REGION 1..34: note = MBD2_A27C
KAFIVTDEDIRKQEERVQQVRKKLEECLMADILS

SEQ ID NO: 3 - protein, 34 aa, synthetic construct
  REGION 1..34: note = MBD2_T6C
KAFIVCDEDIRKQEERVQQVRKKLEEALMADILS

SEQ ID NO: 4 - protein, 34 aa, synthetic construct
  REGION 1..34: note = MBD2_R16C
KAFIVTDEDIRKQEECVQQVRKKLEEALMADILS

SEQ ID NO: 5 - protein, 34 aa, synthetic construct
  REGION 1..34: note = MBD2_V20C
KAFIVTDEDIRKQEERVQQCRKKLEEALMADILS

SEQ ID NO: 6 - protein, 41 aa, synthetic construct
  REGION 1..41: note = p66a_wild type
PEERERMIKQLKEELRLEEAKLVLLKKLRQSQIQKEATAQK

SEQ ID NO: 7 - protein, 41 aa, synthetic construct
  REGION 1..41: note = p66a_I8C
PEERERMCKQLKEELRLEEAKLVLLKKLRQSQIQKEATAQK

SEQ ID NO: 8 - protein, 41 aa, synthetic construct
  REGION 1..41: note = p66a_R29C
PEERERMIKQLKEELRLEEAKLVLLKKLCQSQIQKEATAQK

SEQ ID NO: 9 - protein, 41 aa, synthetic construct
  REGION 1..41: note = p66a_E18C
PEERERMIKQLKEELRLCEAKLVLLKKLRQSQIQKEATAQK

SEQ ID NO: 10 - protein, 41 aa, synthetic construct
  REGION 1..41: note = p66a_L11C
PEERERMIKQCKEELRLEEAKLVLLKKLRQSQIQKEATAQK